European Patent Application EP 4 115 892 A1, published January 11, 2023. Title: IN VITRO METHOD FOR IMPROVING THE PRODUCTION OF EXOSOMES FROM CAR-T CELLS. Applicant: FUNDACION PUBLICA ANDALUZA PROGRESO Y SALUD UNIVERSIDAD DE GRANADA. The sequence listing filed with the application follows.

SEQUENCE LISTING (5 sequences)

SEQ ID NO: 1 - DNA, 20 bp, Artificial sequence
  Artificial sequence
aagtcaacttcaatgtcgga

SEQ ID NO: 2 - DNA, 20 bp, Artificial sequence
  Artificial sequence
actcacgctggatagcctcc

SEQ ID NO: 3 - DNA, 20 bp, Artificial sequence
  Artificial sequence
ggtacggctgacgcagaccg

SEQ ID NO: 4 - DNA, 22 bp, Artificial sequence
  Artificial sequence
gagcatcctggtgaggaataac

SEQ ID NO: 5 - DNA, 20 bp, Artificial sequence
  Artificial sequence
cgcagattcatgaacacggt